European Patent Application EP 4 663 753 A1, published December 17, 2025. Title: TRANSPOSASE, TRANSPOSON, TRANSPOSON SYSTEM, AND USE THEREOF. Applicant: MAXIRNA (SHANGHAI) PHARMACEUTICAL CO.,LTD. The sequence listing filed with the application follows.

SEQUENCE LISTING (61 sequences)

SEQ ID NO: 1 - protein, 425 aa, synthetic construct
MAPTKRHAYNAEFKLKAISHAQEHGNRAAAREFNINESMVRKWRKYEDELRQVKKTTQSFRGNKARWPQLEDKVEQWVAEQRAASRSVSTVTIRMKAIALAREHNISEFRGGPSWCFRFMKRRHLSIRTRTTVSQQLPADYQEKLATFRTYCRNKITEKKIQPEHIINMDEVPLTFDIPVNRTVDKTGARTVNIRTTGNEKTSFTVVLACQANGHKLPPMVIFKRKTLPKENFPAGIVIKANSKGWMDEEKMSEWLREIYVKRPGGFFHTAPSLLIYDSMRAHITEHVKKQVKHTNSVLAVIPGGLTKELQPLDVGVNRAFKARLRTAWEQWMTEGEHTFTKTGRQRRTTYANICKWIVNAWAGISVTTVVRAFRKAGIVTELPDNSSDTDSVNDDFDKTEPGVLDAAIAQLFNSDTEEEVFEGF

SEQ ID NO: 2 - DNA, 28 bp, synthetic construct
  source 1..28: mol_type = other DNA
ccgtattttccgcactataaggcgcacc

SEQ ID NO: 3 - DNA, 28 bp, synthetic construct
  source 1..28: mol_type = other DNA
ggtgcgccttatagtgcggaaaatacgg

SEQ ID NO: 4 - DNA, 28 bp, synthetic construct
  source 1..28: mol_type = other DNA
ccgtattttccgcactataagacgcacc

SEQ ID NO: 5 - DNA, 28 bp, synthetic construct
  source 1..28: mol_type = other DNA
ccgtattttccgcagtataaggcgcacc

SEQ ID NO: 6 - DNA, 28 bp, synthetic construct
  source 1..28: mol_type = other DNA
ccgtattttccggactataaggcgcacc

SEQ ID NO: 7 - DNA, 28 bp, synthetic construct
  source 1..28: mol_type = other DNA
ccgtattttccgcactataaggcgcacc

SEQ ID NO: 8 - DNA, 28 bp, synthetic construct
  source 1..28: mol_type = other DNA
ccgtatatcgcggcgtataagtcgacct

SEQ ID NO: 9 - DNA, 28 bp, synthetic construct
  source 1..28: mol_type = other DNA
ccgtattttccggactataaggcgcact

SEQ ID NO: 10 - DNA, 28 bp, synthetic construct
  source 1..28: mol_type = other DNA
ccgtattttccgcactataaggcgcacc

SEQ ID NO: 11 - DNA, 28 bp, synthetic construct
  source 1..28: mol_type = other DNA
ccgtattttcacgaccataaggcgcact

SEQ ID NO: 12 - DNA, 28 bp, synthetic construct
  source 1..28: mol_type = other DNA
ccgtattttcacgaccataaggcgcact

SEQ ID NO: 13 - DNA, 28 bp, synthetic construct
  source 1..28: mol_type = other DNA
ccgtattttcacaaccataaggcgcgcc

SEQ ID NO: 14 - DNA, 29 bp, synthetic construct
  source 1..29: mol_type = other DNA
ccgtatttttcgctttataggacgcacct

SEQ ID NO: 15 - DNA, 24 bp, synthetic construct
  source 1..24: mol_type = other DNA
ccgtgtttccccgaaaataagaca

SEQ ID NO: 16 - DNA, 27 bp, synthetic construct
  source 1..27: mol_type = other DNA
ccgtattttccggcgtataagacgact

SEQ ID NO: 17 - DNA, 25 bp, synthetic construct
  source 1..25: mol_type = other DNA
ccgtatttttccgtgtataagacgc

SEQ ID NO: 18 - DNA, 26 bp, synthetic construct
  source 1..26: mol_type = other DNA
ctgtattttccggcgtataagacaac

SEQ ID NO: 19 - DNA, 24 bp, synthetic construct
  source 1..24: mol_type = other DNA
ccgtatttgccggcgtataagacg

SEQ ID NO: 20 - DNA, 27 bp, synthetic construct
  source 1..27: mol_type = other DNA
ccgtatattccggcttataagatgact

SEQ ID NO: 21 - DNA, 24 bp, synthetic construct
  source 1..24: mol_type = other DNA
ccgtgtttcctcatatataagaca

SEQ ID NO: 22 - DNA, 27 bp, synthetic construct
  source 1..27: mol_type = other DNA
ctgtatttatgctaatctaatgcgcat

SEQ ID NO: 23 - DNA, 28 bp, synthetic construct
  source 1..28: mol_type = other DNA
ccgtatttttcggaccataagacgcacc

SEQ ID NO: 24 - DNA, 28 bp, synthetic construct
  source 1..28: mol_type = other DNA
ccgtatttactcatgtagaagtcgacct

SEQ ID NO: 25 - DNA, 25 bp, synthetic construct
  source 1..25: mol_type = other DNA
ccgtaaagtctggtgtatagcacgc

SEQ ID NO: 26 - DNA, 28 bp, synthetic construct
  source 1..28: mol_type = other DNA
ctgtaaaatcccgagtataagctgcagc

SEQ ID NO: 27 - DNA, 26 bp, synthetic construct
  source 1..26: mol_type = other DNA
ccgtaaatgttcaaataaaagcccgg

SEQ ID NO: 28 - protein, 31 aa, synthetic construct
TQQKVLELTSDNDRLRKRVEQLSRELDTLRG

SEQ ID NO: 29 - protein, 29 aa, synthetic construct
LQNKVQRLEEQNLSLLDQLRKLQAMVIEI

SEQ ID NO: 30 - protein, 21 aa, synthetic construct
KDVLSEKEKKLEEYKQKLARV

SEQ ID NO: 31 - protein, 36 aa, synthetic construct
LKENQITIRAAFLEKENTALRTEVAELRKEVGKCKT

SEQ ID NO: 32 - DNA, 64 bp, synthetic construct
  source 1..64: mol_type = other DNA
tatatataccgtattttccgcactataagacgcaccccgtattttccgcactataagacgcacc

SEQ ID NO: 33 - DNA, 4974 bp, synthetic construct
  source 1..4974: mol_type = other DNA
aacgccagcaacgcggcctttttacggttcctggccttttgctggccttttgctcacatgttctttcctgcgttatcccctgattctgtggataaccgtattaccgcctttgagtgagctgataccgctcgccgcagccgaacgaccgagcgcagcgagtcagtgagcgaggaagcggaagagcgcccaatacgcaaaccgcctctccccgcgcgttggccgattcattaatgcagctgactgagctcaatgggaaagtaccgttcggagttccgcgttacataacttacggtaaatggcccgcctggctgaccgcccaacgacccccgcccattgacgtcaataatgacgtatgttcccatagtaacgccaatagggactttccattgacgtcaatgggtggagtatttacggtaaactgcccacttggcagtacatcaagtgtatcatatgccaagtacgccccctattgacgtcaatgacggtaaatggcccgcctggcattatgcccagtacatgaccttatgggactttcctacttggcagtacatctacgtattagtcatcgctattaccaaaggatctgcgatcgctccggtgcccgtcagtgggcagagcgcacatcgcccacagtccccgagaagttggggggaggggtcggcaattgaacgggtgcctagagaaggtggcgcggggtaaactgggaaagtgatgtcgtgtactggctccgcctttttcccgagggtgggggagaaccgtatataagtgcagtagtcgccgtgaacgttctttttcgcaacgggtttgccgccagaacacagctgaagcttcgaggggctcgcatctctccttcacgcgcccgccgccctacctgaggccgccatccacgccggttgagtcgcgttctgccgcctcccgcctgtggtgcctcctgaactgcgtccgccgtctaggtaagtttaaagctcaggtcgagaccgggcctttgtccggcgctcccttggagcctacctagactcagccggctctccacgctttgcctgaccctgcttgctcaactctacgtctttgtttcgttttctgttctgcgccgttacagatccaagctgtgaccggcgcctacgaattcaattcataacttcgtatagcatacattatacgaagttatactagtgccaccatcctgctgccaagagggtcaagttggacgcccccaccaagagacacgcctacaacgccgagttcaagctgaaggccatcagccacgcccaggagcacggcaacagagccgccgccagagagttcaacatcaacgagagcatggtgagaaagtggagaaagtacgaggacgagctgagacaggtgaagaagaccacccagagcttcagaggcaacaaggccaggtggccccagctggaggacaaggtggagcagtgggtggccgagcagagagccgccagcagaagcgtgagcaccgtgaccatcagaatgaaggccatcgccctggccagagagcacaacatcagcgagttcagaggcggccccagctggtgcttcagattcatgaagagaagacacctgagcatcagaaccagaaccaccgtgagccagcagctgcccgccgactaccaggagaagctggccaccttcagaacctactgcagaaacaagatcaccgagaagaagatccagcccgagcacatcatcaacatggacgaggtgcccctgaccttcgacatccccgtgaacagaaccgtggacaagaccggcgccagaaccgtgaacatcagaaccaccggcaacgagaagaccagcttcaccgtggtgctggcctgccaggccaacggccacaagctgccccctatggtgatcttcaagagaaagaccctgcccaaggagaacttccccgccggcatcgtgatcaaggccaacagcaagggctggatggacgaggagaagatgagcgagtggctgagagagatctacgtgaagagacccggcggcttcttccacaccgcccccagcctgctgatctacgacagcatgagagcccacatcaccgagcacgtgaagaagcaggtgaagcacaccaacagcgtgctggccgtgatccccggcggcctgaccaaggagctgcagcccctggacgtgggcgtgaacagagccttcaaggccagactgagaaccgcctgggagcagtggatgaccgagggcgagcacaccttcaccaagaccggcagacagagaagaaccacctacgccaacatctgcaagtggatcgtgaacgcctgggccggcatcagcgtgaccaccgtggtgagagccttcagaaaggccggcatcgtgaccgagctgcccgacaacagcagcgacaccgacagcgtgaacgacgacttcgacaagaccgagcccggcgtgctggacgccgccatcgcccagctgttcaacagcgacaccgaggaggaggtgttcgagggcttctgataaggatccgctagcataacttcgtatagcatacattatacgaagttataacttgtttattgcagcttataatggttacaaataaagcaatagcatcacaaatttcacaaataaagcatttttttcactgcattctagttgtggtttgtccaaactcatcaatgtatcttatcatgtctggatcttagtcagttactcgagactggtacctgactggcgtaatagcgaagaggcccgcaccgatcgcccttcccaacagttgcgcagcctgaatggcgaatggaaattgtaagcgttaatattttgttaaaattcgcgttaaatttttgttaaatcagctcattttttaaccaataggccgaaatcggcaaaatcccttataaatcaaaagaatagaccgagatagggttgagtgttgttccagtttggaacaagagtccactattaaagaacgtggactccaacgtcaaagggcgaaaaaccgtctatcagggcgatggcccactacgtgaaccatcaccctaatcaagttttttggggtcgaggtgccgtaaagcactaaatcggaaccctaaagggagcccccgatttagagcttgacggggaaagccggcgaacgtggcgagaaaggaagggaagaaagcgaaaggagcgggcgctagggcgctggcaagtgtagcggtcacgctgcgcgtaaccaccacacccgccgcgcttaatgcgccgctacagggcgcgtcaggtggcacttttcggggaaatgtgcgcggaacccctatttgtttatttttctaaatacattcaaatatgtatccgctcatgagacaataaccctgataaatgcttcaataatattgaaaaaggaagagtatgagtattcaacatttccgtgtcgcccttattcccttttttgcggcattttgccttcctgtttttgctcacccagaaacgctggtgaaagtaaaagatgctgaagatcagttgggtgcacgagtgggttacatcgaactggatctcaacagcggtaagatccttgagagttttcgccccgaagaacgttttccaatgatgagcacttttaaagttctgctatgtggcgcggtattatcccgtattgacgccgggcaagagcaactcggtcgccgcatacactattctcagaatgacttggttgagtactcaccagtcacagaaaagcatcttacggatggcatgacagtaagagaattatgcagtgctgccataaccatgagtgataacactgcggccaacttacttctgacaacgatcggaggaccgaaggagctaaccgcttttttgcacaacatgggggatcatgtaactcgccttgatcgttgggaaccggagctgaatgaagccataccaaacgacgagcgtgacaccacgatgcctgtagcaatggcaacaacgttgcgcaaactattaactggcgaactacttactctagcttcccggcaacaattaatagactggatggaggcggataaagttgcaggaccacttctgcgctcggcccttccggctggctggtttattgctgataaatctggagccggtgagcgtgggtctcgcggtatcattgcagcactggggccagatggtaagccctcccgtatcgtagttatctacacgacggggagtcaggcaactatggatgaacgaaatagacagatcgctgagataggtgcctcactgattaagcattggtaactgtcagaccaagtttactcatatatactttagattgatttaaaacttcatttttaatttaaaaggatctaggtgaagatcctttttgataatctcatgaccaaaatcccttaacgtgagttttcgttccactgagcgtcagaccccgtagaaaagatcaaaggatcttcttgagatcctttttttctgcgcgtaatctgctgcttgcaaacaaaaaaaccaccgctaccagcggtggtttgtttgccggatcaagagctaccaactctttttccgaaggtaactggcttcagcagagcgcagataccaaatactgtccttctagtgtagccgtagttaggccaccacttcaagaactctgtagcaccgcctacatacctcgctctgctaatcctgttaccagtggctgctgccagtggcgataagtcgtgtcttaccgggttggactcaagacgatagttaccggataaggcgcagcggtcgggctgaacggggggttcgtgcacacagcccagcttggagcgaacgacctacaccgaactgagatacctacagcgtgagctatgagaaagcgccacgcttcccgaagggagaaaggcggacaggtatccggtaagcggcagggtcggaacaggagagcgcacgagggagcttccagggggaaacgcctggtatctttatagtcctgtcgggtttcgccacctctgacttgagcgtcgatttttgtgatgctcgtcaggggggcggagcctatggaaa

SEQ ID NO: 34 - DNA, 93 bp, synthetic construct
  source 1..93: mol_type = other DNA
acgcagcagaaggtgctggagctgaccagtgacaatgaccgcctgcgcaagcgggtggaacagctgagccgcgaactggacacgctgcggggc

SEQ ID NO: 35 - DNA, 87 bp, synthetic construct
  source 1..87: mol_type = other DNA
ctgcagaacaaggtgcagcgcctggaggagcagaacctgagcctgctggaccagctgcgcaagctgcaggccatggtgatcgagatc

SEQ ID NO: 36 - DNA, 63 bp, synthetic construct
  source 1..63: mol_type = other DNA
aaggacgtgctgagcgagaaggagaagaagctggaggagtacaagcagaagctggcccgcgtg

SEQ ID NO: 37 - DNA, 108 bp, synthetic construct
  source 1..108: mol_type = other DNA
ctgaaagagaatcagatcaccatccgggcagccttcctggagaaggagaacacagccctgcggacggaggtggccgagctacgcaaggaggtgggcaagtgcaagacc

SEQ ID NO: 38 - DNA, 4935 bp, synthetic construct
  source 1..4935: mol_type = other DNA
gcccctgcagccgaattatattatttttgccaaataatttttaacaaaagctctgaagtcttcttcatttaaattcttagatgatacttcatctggaaaattgtcccaattagtagcatcacgctgtgagtaagttctaaaccatttttttattgttgtattatctctaatcttactactcgatgagttttcggtattatctctatttttaacttggagcaggttccattcattgtttttttcatcatagtgaataaaatcaactgctttaacacttgtgcctgaacaccatatccatccggcgtaatacgactcactatagggagagcggccgccagatcttccggatggctcgagtttttcagcaagattaccgtattttccgcactataaggcgcacctcgcgagtcgacattgattattgactagtcagcaaccaaggatctgcgatcgctccggtgcccgtcagtgggcagagcgcacatcgcccacagtccccgagaagttggggggaggggtcggcaattgaacgggtgcctagagaaggtggcgcggggtaaactgggaaagtgatgtcgtgtactggctccgcctttttcccgagggtgggggagaaccgtatataagtgcagtagtcgccgtgaacgttctttttcgcaacgggtttgccgccagaacacagctgaagcttcgaggggctcgcatctctccttcacgcgcccgccgccctacctgaggccgccatccacgccggttgagtcgcgttctgccgcctcccgcctgtggtgcctcctgaactgcgtccgccgtctaggtaagtttatagctcaggtcgagaccgggcctttgtccggcgctcccttggagcctacctagactcagccggctctccacgctttgcctgaccctgcttgctcaactctacgtctttgtttcgttttctgttctgcgccgttacagatccaagctgtgaccggcgcctacgaattctgcagtcgacggtaccgcgggcccgggatccaccggtcgccaccatggtgagcaagggcgaggagctgttcaccggggtggtgcccatcctggtcgagctggacggcgacgtaaacggccacaagttcagcgtgtccggcgagggcgagggcgatgccacctacggcaagctgaccctgaagttcatctgcaccaccggcaagctgcccgtgccctggcccaccctcgtgaccaccctgacctacggcgtgcagtgcttcagccgctaccccgaccacatgaagcagcacgacttcttcaagtccgccatgcccgaaggctacgtccaggagcgcaccatcttcttcaaggacgacggcaactacaagacccgcgccgaggtgaagttcgagggcgacaccctggtgaaccgcatcgagctgaagggcatcgacttcaaggaggacggcaacatcctggggcacaagctggagtacaactacaacagccacaacgtctatatcatggccgacaagcagaagaacggcatcaaggtgaacttcaagatccgccacaacatcgaggacggcagcgtgcagctcgccgaccactaccagcagaacacccccatcggcgacggccccgtgctgctgcccgacaaccactacctgagcacccagtccgccctgagcaaagaccccaacgagaagcgcgatcacatggtcctgctggagttcgtgaccgccgccgggatcactctcggcatggacgagctgtacaagtaaagcggccgcactcctcaggtgcaggctgcctatcagaaggtggtggctggtgtggccaatgccctggctcacaaataccactgagatctttttccctctgccaaaaattatggggacatcatgaagccccttgagcatctgacttctggctaataaaggaaatttattttcattgcaatagtgtgttggaattttttgtgtctctcactcggaaggacatatgggagggcaaatcatttaaaacatcagaatgagtatttggtttagagtttggcaacatatgcccatatgctggctgccatgaacaaaggtggctataaagaggtcatcagtatatgaaacagccccctgctgtccattccttattccatagaaaagccttgacttgaggttagattttttttatattttgttttgtgttatttttttctttaacatccctaaaattttccttacatgttttactagccagatttttcctcctctcctgactactcccagtcatagctgtccctcttctcttatgaagatccctcgacctcgcgaggtgcgccttatagtgcggaaaatacggtaatctttctagaagatctcctacaatattctcagctgccatggaaaatcgatgttcttcttttattctctcaagattttcaggctgtatattaaaacttatattaagaactatgctaaccacctcatcaggaaccgttgtaggtggcgtgggttttcttggcaatcgactctcatgaaaactacgagctaaatattcaatatgttcctcttgaccaactttattctgcattttttttgaacgaggtttagagcaagcttcaggaaactgagacaggaattttattaaaaatttaaattttgaagaaagttcagggttaatagcatccattttttgctttgcaagttcctcagcattcttaacaaaagacgtctcttttgacatgtttaaagtttaaacctcctgtgtgaaattgttatccgctcacaattccacacattatacgagccggaagcataaagtgtaaagcctggggtgcctaatgagtgagctaactcacattaattgcgttgcgctcactgccaattgctttccagtcgggaaacctgtcgtgccagctgcattaatgaatcggccaacgcgcggggagaggcggtttgcgtattgggcgctcttccgcttcctcgctcactgactcgctgcgctcggtcgttcggctgcggcgagcggtatcagctcactcaaaggcggtaatacggttatccacagaatcaggggataacgcaggaaagaacatgtgagcaaaaggccagcaaaaggccaggaaccgtaaaaaggccgcgttgctggcgtttttccataggctccgcccccctgacgagcatcacaaaaatcgacgctcaagtcagaggtggcgaaacccgacaggactataaagataccaggcgtttccccctggaagctccctcgtgcgctctcctgttccgaccctgccgcttaccggatacctgtccgcctttctcccttcgggaagcgtggcgctttctcatagctcacgctgtaggtatctcagttcggtgtaggtcgttcgctccaagctgggctgtgtgcacgaaccccccgttcagcccgaccgctgcgccttatccggtaactatcgtcttgagtccaacccggtaagacacgacttatcgccactggcagcagccactggtaacaggattagcagagcgaggtatgtaggcggtgctacagagttcttgaagtggtggcctaactacggctacactagaaggacagtatttggtatctgcgctctgctgaagccagttaccttcggaaaaagagttggtagctcttgatccggcaaacaaaccaccgctggtagcggtggtttttttgtttgcaagcagcagattacgcgcagaaaaaaaggatctcaagaagatcctttgatcttttctacggggtctgacgctcagtggaacgaaaactcacgttaagggattttggtcatgagattatcaaaaaggatcttcacctagatccttttaaattaaaaatgaagttttaaatcaatctaaagtatatatgagtaaacttggtctgacagttaccaatgcttaatcagtgaggcacctatctcagcgatctgtctatttcgttcatccatagttgcctgactccccgtcgtgtagataactacgatacgggagggcttaccatctggccccagtgctgcaatgataccgcgagacccacgctcaccggctccagatttatcagcaataaaccagccagccggaagggccgagcgcagaagtggtcctgcaactttatccgcctccatccagtctattaattgttgccgggaagctagagtaagtagttcgccagttaatagtttgcgcaacgttgttgccattgctacaggcatcgtggtgtcacgctcgtcgtttggtatggcttcattcagctccggttcccaacgatcaaggcgagttacatgatcccccatgttgtgcaaaaaagcggttagctccttcggtcctccgatcgttgtcagaagtaagttggccgcagtgttatcactcatggttatggcagcactgcataattctcttactgtcatgccatccgtaagatgcttttctgtgactggtgagtactcaaccaagtcattctgagaatagtgtatgcggcgaccgagttgctcttgcccggcgtcaatacgggataataccgcgccacatagcagaactttaaaagtgctcatcattggaaaacgttcttcggggcgaaaactctcaaggatcttaccgctgttgagatccagttcgatgtaacccactcgtgcacccaactgatcttcagcatcttttactttcaccagcgtttctgggtgagcaaaaacaggaaggcaaaatgccgcaaaaaagggaataagggcgacacggaaatgttgaatactcatactcttcctttttcaatattattgaagcatttatcagggttattgtctcatgagcggatacatatttgaatgtatttagaaaaataaacaaataggggttccgcgcacatttccccgaaaagtgccacctgacgtctaagaaaccattattatcatgacattaacctataaaaataggcgtatcacgaggcccc

SEQ ID NO: 39 - DNA, 5071 bp, synthetic construct
  source 1..5071: mol_type = other DNA
aacgccagcaacgcggcctttttacggttcctggccttttgctggccttttgctcacatgttctttcctgcgttatcccctgattctgtggataaccgtattaccgcctttgagtgagctgataccgctcgccgcagccgaacgaccgagcgcagcgagtcagtgagcgaggaagcggaagagcgcccaatacgcaaaccgcctctccccgcgcgttggccgattcattaatgcagctgactgagctcaatgggaaagtaccgttcggagttccgcgttacataacttacggtaaatggcccgcctggctgaccgcccaacgacccccgcccattgacgtcaataatgacgtatgttcccatagtaacgccaatagggactttccattgacgtcaatgggtggagtatttacggtaaactgcccacttggcagtacatcaagtgtatcatatgccaagtacgccccctattgacgtcaatgacggtaaatggcccgcctggcattatgcccagtacatgaccttatgggactttcctacttggcagtacatctacgtattagtcatcgctattaccaaaggatctgcgatcgctccggtgcccgtcagtgggcagagcgcacatcgcccacagtccccgagaagttggggggaggggtcggcaattgaacgggtgcctagagaaggtggcgcggggtaaactgggaaagtgatgtcgtgtactggctccgcctttttcccgagggtgggggagaaccgtatataagtgcagtagtcgccgtgaacgttctttttcgcaacgggtttgccgccagaacacagctgaagcttcgaggggctcgcatctctccttcacgcgcccgccgccctacctgaggccgccatccacgccggttgagtcgcgttctgccgcctcccgcctgtggtgcctcctgaactgcgtccgccgtctaggtaagtttaaagctcaggtcgagaccgggcctttgtccggcgctcccttggagcctacctagactcagccggctctccacgctttgcctgaccctgcttgctcaactctacgtctttgtttcgttttctgttctgcgccgttacagatccaagctgtgaccggcgcctacgaattcaattcataacttcgtatagcatacattatacgaagttatactagtgccaccatgacgcagcagaaggtgctggagctgaccagtgacaatgaccgcctgcgcaagcgggtggaacagctgagccgcgaactggacacgctgcggggcggccctgctgccaagagggtcaagttggacgcccccaccaagagacacgcctacaacgccgagttcaagctgaaggccatcagccacgcccaggagcacggcaacagagccgccgccagagagttcaacatcaacgagagcatggtgagaaagtggagaaagtacgaggacgagctgagacaggtgaagaagaccacccagagcttcagaggcaacaaggccaggtggccccagctggaggacaaggtggagcagtgggtggccgagcagagagccgccagcagaagcgtgagcaccgtgaccatcagaatgaaggccatcgccctggccagagagcacaacatcagcgagttcagaggcggccccagctggtgcttcagattcatgaagagaagacacctgagcatcagaaccagaaccaccgtgagccagcagctgcccgccgactaccaggagaagctggccaccttcagaacctactgcagaaacaagatcaccgagaagaagatccagcccgagcacatcatcaacatggacgaggtgcccctgaccttcgacatccccgtgaacagaaccgtggacaagaccggcgccagaaccgtgaacatcagaaccaccggcaacgagaagaccagcttcaccgtggtgctggcctgccaggccaacggccacaagctgccccctatggtgatcttcaagagaaagaccctgcccaaggagaacttccccgccggcatcgtgatcaaggccaacagcaagggctggatggacgaggagaagatgagcgagtggctgagagagatctacgtgaagagacccggcggcttcttccacaccgcccccagcctgctgatctacgacagcatgagagcccacatcaccgagcacgtgaagaagcaggtgaagcacaccaacagcgtgctggccgtgatccccggcggcctgaccaaggagctgcagcccctggacgtgggcgtgaacagagccttcaaggccagactgagaaccgcctgggagcagtggatgaccgagggcgagcacaccttcaccaagaccggcagacagagaagaaccacctacgccaacatctgcaagtggatcgtgaacgcctgggccggcatcagcgtgaccaccgtggtgagagccttcagaaaggccggcatcgtgaccgagctgcccgacaacagcagcgacaccgacagcgtgaacgacgacttcgacaagaccgagcccggcgtgctggacgccgccatcgcccagctgttcaacagcgacaccgaggaggaggtgttcgagggcttctgataaggatccgctagcataacttcgtatagcatacattatacgaagttataacttgtttattgcagcttataatggttacaaataaagcaatagcatcacaaatttcacaaataaagcatttttttcactgcattctagttgtggtttgtccaaactcatcaatgtatcttatcatgtctggatcttagtcagttactcgagactggtacctgactggcgtaatagcgaagaggcccgcaccgatcgcccttcccaacagttgcgcagcctgaatggcgaatggaaattgtaagcgttaatattttgttaaaattcgcgttaaatttttgttaaatcagctcattttttaaccaataggccgaaatcggcaaaatcccttataaatcaaaagaatagaccgagatagggttgagtgttgttccagtttggaacaagagtccactattaaagaacgtggactccaacgtcaaagggcgaaaaaccgtctatcagggcgatggcccactacgtgaaccatcaccctaatcaagttttttggggtcgaggtgccgtaaagcactaaatcggaaccctaaagggagcccccgatttagagcttgacggggaaagccggcgaacgtggcgagaaaggaagggaagaaagcgaaaggagcgggcgctagggcgctggcaagtgtagcggtcacgctgcgcgtaaccaccacacccgccgcgcttaatgcgccgctacagggcgcgtcaggtggcacttttcggggaaatgtgcgcggaacccctatttgtttatttttctaaatacattcaaatatgtatccgctcatgagacaataaccctgataaatgcttcaataatattgaaaaaggaagagtatgagtattcaacatttccgtgtcgcccttattcccttttttgcggcattttgccttcctgtttttgctcacccagaaacgctggtgaaagtaaaagatgctgaagatcagttgggtgcacgagtgggttacatcgaactggatctcaacagcggtaagatccttgagagttttcgccccgaagaacgttttccaatgatgagcacttttaaagttctgctatgtggcgcggtattatcccgtattgacgccgggcaagagcaactcggtcgccgcatacactattctcagaatgacttggttgagtactcaccagtcacagaaaagcatcttacggatggcatgacagtaagagaattatgcagtgctgccataaccatgagtgataacactgcggccaacttacttctgacaacgatcggaggaccgaaggagctaaccgcttttttgcacaacatgggggatcatgtaactcgccttgatcgttgggaaccggagctgaatgaagccataccaaacgacgagcgtgacaccacgatgcctgtagcaatggcaacaacgttgcgcaaactattaactggcgaactacttactctagcttcccggcaacaattaatagactggatggaggcggataaagttgcaggaccacttctgcgctcggcccttccggctggctggtttattgctgataaatctggagccggtgagcgtgggtctcgcggtatcattgcagcactggggccagatggtaagccctcccgtatcgtagttatctacacgacggggagtcaggcaactatggatgaacgaaatagacagatcgctgagataggtgcctcactgattaagcattggtaactgtcagaccaagtttactcatatatactttagattgatttaaaacttcatttttaatttaaaaggatctaggtgaagatcctttttgataatctcatgaccaaaatcccttaacgtgagttttcgttccactgagcgtcagaccccgtagaaaagatcaaaggatcttcttgagatcctttttttctgcgcgtaatctgctgcttgcaaacaaaaaaaccaccgctaccagcggtggtttgtttgccggatcaagagctaccaactctttttccgaaggtaactggcttcagcagagcgcagataccaaatactgtccttctagtgtagccgtagttaggccaccacttcaagaactctgtagcaccgcctacatacctcgctctgctaatcctgttaccagtggctgctgccagtggcgataagtcgtgtcttaccgggttggactcaagacgatagttaccggataaggcgcagcggtcgggctgaacggggggttcgtgcacacagcccagcttggagcgaacgacctacaccgaactgagatacctacagcgtgagctatgagaaagcgccacgcttcccgaagggagaaaggcggacaggtatccggtaagcggcagggtcggaacaggagagcgcacgagggagcttccagggggaaacgcctggtatctttatagtcctgtcgggtttcgccacctctgacttgagcgtcgatttttgtgatgctcgtcaggggggcggagcctatggaaa

SEQ ID NO: 40 - DNA, 4735 bp, synthetic construct
  source 1..4735: mol_type = other DNA
gcccctgcagccgaattatattatttttgccaaataatttttaacaaaagctctgaagtcttcttcatttaaattcttagatgatacttcatctggaaaattgtcccaattagtagcatcacgctgtgagtaagttctaaaccatttttttattgttgtattatctctaatcttactactcgatgagttttcggtattatctctatttttaacttggagcaggttccattcattgtttttttcatcatagtgaataaaatcaactgctttaacacttgtgcctgaacaccatatccatccggcgtaatacgactcactatagggagagcggccgccagatcttccggatggctcgagtttttcagcaagatggatcctaccgtattttccgcactataaggcgcacctcgcgagcttggctgcaggtcgtcgaaattctaccgggtaggggaggcgcttttcccaaggcagtctggagcatgcgctttagcagccccgctgggcacttggcgctacacaagtggcctctggcctcgcacacattccacatccaccggtaggcgccaaccggctccgttctttggtggccccttcgcgccaccttctactcctcccctagtcaggaagttcccccccgccccgcagctcgcgtcgtgcaggacgtgacaaatggaagtagcacgtctcactagtctcgtgcagatggacagcaccgctgagcaatggaagcgggtaggcctttggggcagcggccaatagcagctttgctccttcgctttctgggctcagaggctgggaaggggtgggtccgggggcgggctcaggggcgggctcaggggcggggcgggcgcccgaaggtcctccggaggcccggcattctgcacgcttcaaaagcgcacgtctgccgcgctgttctcctcttcctcatctccgggcctttcgacctgcagcctgttgacaattaatcatcggcatagtatatcggcatagtataatacgacaaggtgaggaactaaaccctgatatgggatcggccattgaacaagatggattgcacgcaggttctccggccgcttgggtggagaggctattcggctatgactgggcacaacagacaatcggctgctctgatgccgccgtgttccggctgtcagcgcaggggcgcccggttctttttgtcaagaccgacctgtccggtgccctgaatgaactgcaggacgaggcagcgcggctatcgtggctggccacgacgggcgttccttgcgcagctgtgctcgacgttgtcactgaagcgggaagggactggctgctattgggcgaagtgccggggcaggatctcctgtcatctcaccttgctcctgccgagaaagtatccatcatggctgatgcaatgcggcggctgcatacgcttgatccggctacctgcccattcgaccaccaagcgaaacatcgcatcgagcgagcacgtactcggatggaagccggtcttgtcgatcaggatgatctggacgaagagcatcaggggctcgcgccagccgaactgttcgccaggctcaaggcgcgcatgcccgacggcgatgatctcgtcgtgacccatggcgatgcctgcttgccgaatatcatggtggaaaatggccgcttttctggattcatcgactgtggccggctgggtgtggcggaccgctatcaggacatagcgttggctacccgtgatattgctgaagagcttggcggcgaatgggctgaccgcttcctcgtgctttacggtatcgccgctcccgattcgcagcgcatcgccttctatcgccttcttgacgagttcttctgaggggatcaattctctagagctcgctgatcagcctcgactgtgccttctagttgccagccatctgttgtttgcccctcccccgtgccttccttgaccctggaaggtgccactcccactgtcctttcctaataaaatgaggaaattgcatcgcattgtctgagtaggtgtcattctattctggggggtggggtggggcaggacagcaagggggaggattgggaagacaatagcaggcatgctggggatcgtcgcgagcggccgcgaattcggtgcgccttatagtgcggaaaatacggtaggatccatctttctagaagatctcctacaatattctcagctgccatggaaaatcgatgttcttcttttattctctcaagattttcaggctgtatattaaaacttatattaagaactatgctaaccacctcatcaggaaccgttgtaggtggcgtgggttttcttggcaatcgactctcatgaaaactacgagctaaatattcaatatgttcctcttgaccaactttattctgcattttttttgaacgaggtttagagcaagcttcaggaaactgagacaggaattttattaaaaatttaaattttgaagaaagttcagggttaatagcatccattttttgctttgcaagttcctcagcattcttaacaaaagacgtctcttttgacatgtttaaagtttaaacctcctgtgtgaaattgttatccgctcacaattccacacattatacgagccggaagcataaagtgtaaagcctggggtgcctaatgagtgagctaactcacattaattgcgttgcgctcactgccaattgctttccagtcgggaaacctgtcgtgccagctgcattaatgaatcggccaacgcgcggggagaggcggtttgcgtattgggcgctcttccgcttcctcgctcactgactcgctgcgctcggtcgttcggctgcggcgagcggtatcagctcactcaaaggcggtaatacggttatccacagaatcaggggataacgcaggaaagaacatgtgagcaaaaggccagcaaaaggccaggaaccgtaaaaaggccgcgttgctggcgtttttccataggctccgcccccctgacgagcatcacaaaaatcgacgctcaagtcagaggtggcgaaacccgacaggactataaagataccaggcgtttccccctggaagctccctcgtgcgctctcctgttccgaccctgccgcttaccggatacctgtccgcctttctcccttcgggaagcgtggcgctttctcatagctcacgctgtaggtatctcagttcggtgtaggtcgttcgctccaagctgggctgtgtgcacgaaccccccgttcagcccgaccgctgcgccttatccggtaactatcgtcttgagtccaacccggtaagacacgacttatcgccactggcagcagccactggtaacaggattagcagagcgaggtatgtaggcggtgctacagagttcttgaagtggtggcctaactacggctacactagaaggacagtatttggtatctgcgctctgctgaagccagttaccttcggaaaaagagttggtagctcttgatccggcaaacaaaccaccgctggtagcggtggtttttttgtttgcaagcagcagattacgcgcagaaaaaaaggatctcaagaagatcctttgatcttttctacggggtctgacgctcagtggaacgaaaactcacgttaagggattttggtcatgagattatcaaaaaggatcttcacctagatccttttaaattaaaaatgaagttttaaatcaatctaaagtatatatgagtaaacttggtctgacagttaccaatgcttaatcagtgaggcacctatctcagcgatctgtctatttcgttcatccatagttgcctgactccccgtcgtgtagataactacgatacgggagggcttaccatctggccccagtgctgcaatgataccgcgagacccacgctcaccggctccagatttatcagcaataaaccagccagccggaagggccgagcgcagaagtggtcctgcaactttatccgcctccatccagtctattaattgttgccgggaagctagagtaagtagttcgccagttaatagtttgcgcaacgttgttgccattgctacaggcatcgtggtgtcacgctcgtcgtttggtatggcttcattcagctccggttcccaacgatcaaggcgagttacatgatcccccatgttgtgcaaaaaagcggttagctccttcggtcctccgatcgttgtcagaagtaagttggccgcagtgttatcactcatggttatggcagcactgcataattctcttactgtcatgccatccgtaagatgcttttctgtgactggtgagtactcaaccaagtcattctgagaatagtgtatgcggcgaccgagttgctcttgcccggcgtcaatacgggataataccgcgccacatagcagaactttaaaagtgctcatcattggaaaacgttcttcggggcgaaaactctcaaggatcttaccgctgttgagatccagttcgatgtaacccactcgtgcacccaactgatcttcagcatcttttactttcaccagcgtttctgggtgagcaaaaacaggaaggcaaaatgccgcaaaaaagggaataagggcgacacggaaatgttgaatactcatactcttcctttttcaatattattgaagcatttatcagggttattgtctcatgagcggatacatatttgaatgtatttagaaaaataaacaaataggggttccgcgcacatttccccgaaaagtgccacctgacgtctaagaaaccattattatcatgacattaacctataaaaataggcgtatcacgaggcc

SEQ ID NO: 41 - RNA, 1651 nt, synthetic construct
  source 1..1651: mol_type = other RNA
gggaataagaatcaaatagaagtaagtacacaagaaacctcaagaagccaccatgacgcagcagaaggtgctggagctgaccagtgacaatgaccgcctgcgcaagcgggtggaacagctgagccgcgaactggacacgctgcggggcggccctgctgccaagagggtcaagttggacgcccccaccaagagacacgcctacaacgccgagttcaagctgaaggccatcagccacgcccaggagcacggcaacagagccgccgccagagagttcaacatcaacgagagcatggtgagaaagtggagaaagtacgaggacgagctgagacaggtgaagaagaccaagaaggccttcagaggcaacaaggccaggtggccccagctggaggacaaggtggagcagtgggtggccgagcagagagccgccagcagaagcgtgagcaccgtgaccatcagaatgaaggccatcgccctggccagagagcacaacatcagcgagttcagaggcggccccagctggtgcttcagattcatgaagagaagacacctgagcatcagaaccagaaccaccgtgagccagcagctgcccgccgactaccaggagaagctggccaccttcagaacctactgcagaaacaagatcaccgagaagaagatccagcccgagcacatcatcaacatggacgaggtgcccctgaccttcgacatccccgtgaacagaaccgtggacaagaccggcgccagaaccgtgaacatcagaaccaccggcaacgagaagaccagcttcaccgtggtgctggcctgccaggccaacggccacaagctgccccctatggtgatcttcaagagaaagaccctgcccaaggagaacttccccgccggcatcgtgatcaaggccaacagcaagggctggatggacgaggagaagatgagcgagtggctgagagagatctacgtgaagagacccggcggcttcttccacaccgcccccagcctgctgatctacgacagcatgagagcccacatcaccgagcacgtgaagaagcaggtgaagcacaccaacagcgtgctggccgtgatccccggcggcctgaccaaggagctgcagcccctggacgtgggcgtgaacagagccttcaaggccagactgagaaccgcctgggagcagtggatgaccgagggcgagcacaccttcaccaagaccggcagacagagaagaaccacctacgccaacatctgcaagtggatcgtgaacgcctgggccggcatcagcgtgaccaccgtggtgagagccttcagaaaggccggcatcgtgaccgagctgcccgacaacagcagcgacaccgacagcgtgaacgacgacttcgacaagaccgagcccggcgtgctggacgccgccatcgcccagctgttcaacagcgacaccgaggaggaggtgttcgagggcttctgataacttaagtctgacacagacacgttactaacacagttagtaaccactctatcaccgatagacacatgatatcccatatcataagcttaaaaaaaaaaaaaaaaaaaaaaaaaaaaaaaaaaaaaaaaaaaaaaaaaaggaaaaaaaaaaaaaaaaaaaaaaaaaaaaaaaaaaaaaaaaaaaaaaaaaaaaaaaaaa

SEQ ID NO: 42 - DNA, 2726 bp, synthetic construct
  source 1..2726: mol_type = other DNA
ttaggttctgcttttctcaataacctctttggctgaggtgtattcttccagtggttcttctgccattgcctgttcaatcactctcaggattggttctggaatatctgatggggtgctcagcagatattcaatggcttccagggttggttcatcaatatctgaggacacttttctgatgatttccagttttctttcatcagtgctcatgatggccctcctatagtgagttgtattatactatgcagatatactatgccaatgtttaattgtcaacctgcaggaatatataccgtattttccgcactataaggcgcaccccgtattttccgcactataaggcgcacctctagacatcttggaccattagctccacaggtatcttcttccctctagtggtcataacagcagcttcagctacctctctctctgctgccagtagagggcacacttactttactcattcctttaatggtcttttctggacaccactaggggtcagaagtagttcatcaaactttcttccctccctagagtcaatgggaaaaacccattggagccaagtacactgactcaatagggactttccattgggttttgcccagtacataaggtcaatagggggtgagtcaacaggaaagtcccattggagccaagtacattgagtcaatagggactttccaatgggttttgcccagtacataaggtcaatgggaggtaagccaatgggtttttcccattactgacatgtatactgagtcattagggactttccaatgggttttgcccagtacataaggtcaataggggtgaatcaacaggaaagtcccattggagccaagtacactgagtcaatagggactttccattgggttttgcccagtacaaaaggtcaatagggggtgagtcaatgggtttttcccattattggcacatacataaggtcaataggggtgactagtggagaagagcatgcttgagggctgagtgcccctcagtgggcagagagcacatggcccacagtccctgagaagttggggggaggggtgggcaattgaactggtgcctagagaaggtggggcttgggtaaactgggaaagtgatgtggtgtactggctccacctttttccccagggtgggggagaaccatatataagtgcagtagtctctgtgaacattcaagcttctgccttctccctcctgtgagtttggtaagtcactgactgtctatgcctgggaaagggtgggcaggaggtggggcagtgcaggaaaagtggcactgtgaaccctgcagccctagacaattgtactaaccttcttctctttcctctcctgacaggggtctccaattgccaccatggtgagcaagggagaggagctgttcactggggtggtgcccatcctggtggagctggatggagatgtgaatggccacaagttctctgtgtctggagagggagagggagatgccacctatggcaagctgaccctgaagttcatctgcaccacaggcaagctgcctgtgccctggcccaccctggtgaccaccctgacctatggagtgcagtgcttcagcagataccctgaccacatgaagcagcatgacttcttcaagtctgccatgcctgagggctatgtccaggagagaaccatcttcttcaaggatgatggcaactacaagaccagagctgaggtgaagtttgagggagacaccctggtgaacagaattgagctgaagggcattgacttcaaggaggatggcaacatcctggggcacaagctggagtacaactacaacagccacaatgtctatatcatggctgacaagcagaagaatggcatcaaggtgaacttcaagatcagacacaacattgaggatggctctgtgcagctggctgaccactaccagcagaacacccccattggagatggccctgtgctgctgcctgacaaccactacctgagcacccagtctgccctgagcaaggaccccaatgagaagagagatcacatggtcctgctggagtttgtgacagctgctgggatcactctgggcatggatgagctgtacaagtaatgaggatcctaagatacattgatgagtttggacaaaccacaactagaatgcagtgaaaaaaatgctttatttgtgaaatttgtgatgctattgctttatttgtaaccattataagctgcaataaacaagtttagggagggaagaaagtttgatgaactacttctgacccctagtggtgtccagaaaagaccattaaaggaatgagtaaagtaagtgtgccctctactggcagcagagagagaggtagctgaagctgctgttatgaccactagagggaagaagatacctgtggagctaatggtccaagatgcttaagggtgcgccttatagtgcggaaaatacggggtgcgccttatagtgcggaaaatacggtatataagagctcaatcagcagttcaacctgttgatagtatgtactaagctctcatgtttaatgtactaagctctcatgtttaatgaactaaaccctcatggctaatgtactaagctctcatggctaatgtactaagctctcatgtttcatgtactaagctctcatgtttgaacaataaaattaatataaatcagcaacttaaatagcctctaaggttttaagttttataagaaaaaaaagaatatataaggcttttaaaggttttaaggtttcctagct

SEQ ID NO: 43 - DNA, 3716 bp, synthetic construct
  source 1..3716: mol_type = other DNA
tcgacagcactagtgcaggatccttacttgtacagctcatccatgcccagagtgatcccagcagctgtcacaaactccagcaggaccatgtgatctctcttctcattggggtccttgctcagggcagactgggtgctcaggtagtggttgtcaggcagcagcacagggccatctccaatgggggtgttctgctggtagtggtcagccagctgcacagagccatcctcaatgttgtgtctgatcttgaagttcaccttgatgccattcttctgcttgtcagccatgatatagacattgtggctgttgtagttgtactccagcttgtgccccaggatgttgccatcctccttgaagtcaatgcccttcagctcaattctgttcaccagggtgtctccctcaaacttcacctcagctctggtcttgtagttgccatcatccttgaagaagatggttctctcctggacatagccctcaggcatggcagacttgaagaagtcatgctgcttcatgtggtcagggtatctgctgaagcactgcactccataggtcagggtggtcaccagggtgggccagggcacaggcagcttgcctgtggtgcagatgaacttcagggtcagcttgccataggtggcatctccctctccctctccagacacagagaacttgtggccattcacatctccatccagctccaccaggatgggcaccaccccagtgaacagctcctctcccttgctcaccatggtggcaattcgtaggcgccggtcacagcttggatctgtaacggcgcagaacagaaaacgaaacaaagacgtagagttgagcaagcagggtcaggcaaagcgtggagagccggctgagtctaggtaggctccaagggagcgccggacaaaggcccggtctcgacctgagctataaacttacctagacggcggacgcagttcaggaggcaccacaggcgggaggcggcagaacgcgactcaaccggcgtggatggcggcctcaggtagggcggcgggcgcgtgaaggagagatgcgagcccctcgaagcttcagctgtgttctggcggcaaacccgttgcgaaaaagaacgttcacggcgactactgcacttatatacggttctcccccaccctcgggaaaaaggcggagccagtacacgacatcactttcccagtttaccccgcgccaccttctctaggcacccgttcaattgccgacccctccccccaacttctcggggactgtgggcgatgtgcgctctgcccactgacgggcaccggagcgatcgcagatccttggttgctgactaattgagatgcatgctttgcatacttctgcctgctggggagcctggggactttccacacctggttgctgactaattgagatgcatgctttgcatacttctgcctgctggggagcctggggactttccacaccgctagctagggagggaagaaagtttgatgaactacttctgacccctagtggtgtccagaaaagaccattaaaggaatgagtaaagtaagtgtgccctctactggcagcagagagagaggtagctgaagctgctgttatgaccactagagggaagaagatacctgtggagctaatggtccaagatgtctagacatgcgtcaattttacgcagactatctttctagggttaatcgaagagcaaaaggccagcaaaaggccaggaaccgtaaaaaggccgcgttgctggcgtttttccataggctccgcccccctgacgagcatcacaaaaatcgacgctcaagtcagaggtggcgaaacccgacaggactataaagataccaggcgtttccccctggaagctccctcgtgcgctctcctgttccgaccctgccgcttacgggatacctgtccgcctttctcccttcgggaagcgtggcgctttctcatagctcacgctgtaggtatctcagttcggtgtaggtcgttcgctccaagctgggctgtgtgcacgaaccccccgttcagcccgaccgctgcgccttatccggtaactatcgtcttgagtccaacccggtaagacacgacttatcgccactggcagcagccactggtaacaggattagcagagcgaggtatgtaggcggtgctacagagttcttgaagtggtggcctaactacggctacactagaagaacagtatttggtatctgcgctctgctgaagccagttaccttcggaaaaagagttggtagctcttgatccggcaaacaaaccaccgctggtagcggtggtttttttgtttgcaagcagcagattacgcgcagaaaaaaaggatctcaagaagatcctttgatcttttctacggggtctgacgctcagtggaacgaaaactcacggggattttggtcatgccgtctcagaagaactcgtcaagaaggcgatagaaggcgatgcgctgcgaatcgggagcggcgataccgtaaagcacgaggaagcggtcagcccattcgccgccaagctcttcagcaatatcacgggtagccaacgctatgtcctgatagcggtccgccacacccagccggccacagtcgatgaatccagaaaagcggccattttccaccatgatattcggcaagcaggcatcgccatgggtcacgacgagatcctcgccgtcgggcatgctcgccttgagcctggcgaacagttcggctggcgcgagcccctgatgctcttcgtccagatcatcctgatcgacaagaccggcttccatccgagtacgtgctctctcgatgcgatgtttcgcttggtggtcgaatgggcaggtagccggatcaagcgtatgcagccgccgcattgcatcagccatgatggatactttctcggcaggagcaaggtgagatgacaggagatcctgccccggcacttcgcccaatagcagccagtcccttcccgcttcagtgacaacgtcgagtacagctgcgcaaggaacgcccgtcgtggccagccacgatagccgcgctgcctcgtcttgcagttcattcagggcaccggacaggtcggtcttgacaaaaagaaccgggcgcccctgcgctgacagccggaacacggcggcatcagagcagccgattgtctgttgtgcccagtcatagccgaatagcctctccacccaagcggccggagaacctgcgtgcaatccatcttgttcaatcataatattattgaagcatttatcagggttcgtctcgtcccggtctcctcccatgcatgggcgcgccttaaccctagaaagataatcatattgtgacgtacgttaaagataatcatgcgtaaaattgacgcatgcttaagagagaaatgttctggcacctgcacttgcactggggacagcctattttgctagtttgttttgtttcgttttgttttgatggagagcgtatgttagtcatactgattcacacaaaaaaccaacacacagatgtaatgaaaataaagatattttattgatatcccatagagcccaccgcatccccagcatgcctgctattgtcatcccaatcctcccccttgctgtcctgccccaccccaccccccagaatagaatgacacctactcagacaatgcgatgcaatttcctcattttattaggaaaggacagtgggagtggcaccttccagggtcaaggaaggcacgggggaggggcaaacaacagatggctggcaactagaaggcacagg

SEQ ID NO: 44 - DNA, 4116 bp, synthetic construct
  source 1..4116: mol_type = other DNA
aattcgtaggcgccggtcacagcttggatctgtaacggcgcagaacagaaaacgaaacaaagacgtagagttgagcaagcagggtcaggcaaagcgtggagagccggctgagtctaggtaggctccaagggagcgccggacaaaggcccggtctcgacctgagctataaacttacctagacggcggacgcagttcaggaggcaccacaggcgggaggcggcagaacgcgactcaaccggcgtggatggcggcctcaggtagggcggcgggcgcgtgaaggagagatgcgagcccctcgaagcttcagctgtgttctggcggcaaacccgttgcgaaaaagaacgttcacggcgactactgcacttatatacggttctcccccaccctcgggaaaaaggcggagccagtacacgacatcactttcccagtttaccccgcgccaccttctctaggcacccgttcaattgccgacccctccccccaacttctcggggactgtgggcgatgtgcgctctgcccactgacgggcaccggagcgatcgcagatccttggttgctgactaattgagatgcatgctttgcatacttctgcctgctggggagcctggggactttccacacctggttgctgactaattgagatgcatgctttgcatacttctgcctgctggggagcctggggactttccacaccgctagctagggagggaagaaagtttgatgaactacttctgacccctagtggtgtccagaaaagaccattaaaggaatgagtaaagtaagtgtgccctctactggcagcagagagagaggtagctgaagctgctgttatgaccactagagggaagaagatacctgtggagctaatggtccaagatgtctagacatgcgtcaattttacgcagactatctttctagggttaatcgaagagcaaaaggccagcaaaaggccaggaaccgtaaaaaggccgcgttgctggcgtttttccataggctccgcccccctgacgagcatcacaaaaatcgacgctcaagtcagaggtggcgaaacccgacaggactataaagataccaggcgtttccccctggaagctccctcgtgcgctctcctgttccgaccctgccgcttacgggatacctgtccgcctttctcccttcgggaagcgtggcgctttctcatagctcacgctgtaggtatctcagttcggtgtaggtcgttcgctccaagctgggctgtgtgcacgaaccccccgttcagcccgaccgctgcgccttatccggtaactatcgtcttgagtccaacccggtaagacacgacttatcgccactggcagcagccactggtaacaggattagcagagcgaggtatgtaggcggtgctacagagttcttgaagtggtggcctaactacggctacactagaagaacagtatttggtatctgcgctctgctgaagccagttaccttcggaaaaagagttggtagctcttgatccggcaaacaaaccaccgctggtagcggtggtttttttgtttgcaagcagcagattacgcgcagaaaaaaaggatctcaagaagatcctttgatcttttctacggggtctgacgctcagtggaacgaaaactcacggggattttggtcatgccgtctcagaagaactcgtcaagaaggcgatagaaggcgatgcgctgcgaatcgggagcggcgataccgtaaagcacgaggaagcggtcagcccattcgccgccaagctcttcagcaatatcacgggtagccaacgctatgtcctgatagcggtccgccacacccagccggccacagtcgatgaatccagaaaagcggccattttccaccatgatattcggcaagcaggcatcgccatgggtcacgacgagatcctcgccgtcgggcatgctcgccttgagcctggcgaacagttcggctggcgcgagcccctgatgctcttcgtccagatcatcctgatcgacaagaccggcttccatccgagtacgtgctctctcgatgcgatgtttcgcttggtggtcgaatgggcaggtagccggatcaagcgtatgcagccgccgcattgcatcagccatgatggatactttctcggcaggagcaaggtgagatgacaggagatcctgccccggcacttcgcccaatagcagccagtcccttcccgcttcagtgacaacgtcgagtacagctgcgcaaggaacgcccgtcgtggccagccacgatagccgcgctgcctcgtcttgcagttcattcagggcaccggacaggtcggtcttgacaaaaagaaccgggcgcccctgcgctgacagccggaacacggcggcatcagagcagccgattgtctgttgtgcccagtcatagccgaatagcctctccacccaagcggccggagaacctgcgtgcaatccatcttgttcaatcataatattattgaagcatttatcagggttcgtctcgtcccggtctcctcccatgcatgggcgcgccttaaccctagaaagataatcatattgtgacgtacgttaaagataatcatgcgtaaaattgacgcatgcttaagagagaaatgttctggcacctgcacttgcactggggacagcctattttgctagtttgttttgtttcgttttgttttgatggagagcgtatgttagtcatactgattcacacaaaaaaccaacacacagatgtaatgaaaataaagatattttattgatatcccatagagcccaccgcatccccagcatgcctgctattgtcatcccaatcctcccccttgctgtcctgccccaccccaccccccagaatagaatgacacctactcagacaatgcgatgcaatttcctcattttattaggaaaggacagtgggagtggcaccttccagggtcaaggaaggcacgggggaggggcaaacaacagatggctggcaactagaaggcacaggtcgacttatcagcgagggggcagggcctgcatgtgaagggcgtcgtaggtgtccttggtggctgtactgagaccctggtaaaggccatcgtgccccttgcccctccggcgctcgcctttcatcccaatctcactgtaggcctccgccatcttatctttctgcagttcattgtacaggccttcctgagggttcttccttctcggctttccccccatctcagggtcccggccacgtctcttgtccaaaacatcgtactcctctcttcgtcctagattgagctcgttatagagctggttctggccctgctggtacgcgggggcgtctgcgctcctgctgaacttcactctggagcgataggctgcgaagtcgcgtggtggggcatagggctggtaatgcttgcgggtgggcccggggcggcggggagtcatgttcatgtagtcactgtgcaggagcctgctcctcttactcctcacccagaaaataataaaggccactgttactagcaagctatagcaagccaggactccaccaaccaccaccagcacccaaaagggatcacaggcgaagtccagccccctcgtgtgcactgcgccccccgccgctggccggcacgcctctgggcgcagggacaggggctgcgacgcgatggtgggcgccggtgttggtggtcgcggcgctggcgtcgtggtgggcttcgctggcaggaagaccggcacgaagctgctcacggtcacctgggtgccctggccccagtcggggtcgtagtcgttgtagtccttgttgctggcggcgcagtagtacatgccggtgtcctcgggcttcagcatgttcatctgcaggtacagggtgttcttggcgttgtcgcggctgatggtgaagcggcccttcacgctgtcggcgtagtaggtcttgccgccgctgttgatggtggccaccagctggcgctccttctcgctgatctggcggtaccagcccatgtaggcgatgctgatgatgggggtgctggcggcgcagctcaggcgcaggctgccgccggcctgcacgaagccgccgccgctctccaccacctgcacctggctcggcctggcggcgtggagcagcaaggccagcggcaggagcaaggcggtcactggtaaggccatggtggcg

SEQ ID NO: 45 - DNA, 3663 bp, synthetic construct
  source 1..3663: mol_type = other DNA
tcgacctgtgccttctagttgccagccatctgttgtttgcccctcccccgtgccttccttgaccctggaaggtgccactcccactgtcctttcctaataaaatgaggaaattgcatcgcattgtctgagtaggtgtcattctattctggggggtggggtggggcaggacagcaagggggaggattgggatgacaatagcaggcatgctggggatgcggtgggctctatgggatatcaataaaatatctttattttcattacatctgtgtgttggttttttgtgtgaatcagtatgactaacatacgctctccatcaaaacaaaacgaaacaaaacaaactagcaaaataggctgtccccagtgcaagtgcaggtgccagaacatttctctcttaagcatgcgtcaattttacgcatgattatctttaacgtacgtcacaatatgattatctttctagggttaaggcgcgcccatgcatgggaggagaccgggacgagacgaaccctgataaatgcttcaataatattatgattgaacaagatggattgcacgcaggttctccggccgcttgggtggagaggctattcggctatgactgggcacaacagacaatcggctgctctgatgccgccgtgttccggctgtcagcgcaggggcgcccggttctttttgtcaagaccgacctgtccggtgccctgaatgaactgcaagacgaggcagcgcggctatcgtggctggccacgacgggcgttccttgcgcagctgtactcgacgttgtcactgaagcgggaagggactggctgctattgggcgaagtgccggggcaggatctcctgtcatctcaccttgctcctgccgagaaagtatccatcatggctgatgcaatgcggcggctgcatacgcttgatccggctacctgcccattcgaccaccaagcgaaacatcgcatcgagagagcacgtactcggatggaagccggtcttgtcgatcaggatgatctggacgaagagcatcaggggctcgcgccagccgaactgttcgccaggctcaaggcgagcatgcccgacggcgaggatctcgtcgtgacccatggcgatgcctgcttgccgaatatcatggtggaaaatggccgcttttctggattcatcgactgtggccggctgggtgtggcggaccgctatcaggacatagcgttggctacccgtgatattgctgaagagcttggcggcgaatgggctgaccgcttcctcgtgctttacggtatcgccgctcccgattcgcagcgcatcgccttctatcgccttcttgacgagttcttctgagacggcatgaccaaaatccccgtgagttttcgttccactgagcgtcagaccccgtagaaaagatcaaaggatcttcttgagatcctttttttctgcgcgtaatctgctgcttgcaaacaaaaaaaccaccgctaccagcggtggtttgtttgccggatcaagagctaccaactctttttccgaaggtaactggcttcagcagagcgcagataccaaatactgttcttctagtgtagccgtagttaggccaccacttcaagaactctgtagcaccgcctacatacctcgctctgctaatcctgttaccagtggctgctgccagtggcgataagtcgtgtcttaccgggttggactcaagacgatagttaccggataaggcgcagcggtcgggctgaacggggggttcgtgcacacagcccagcttggagcgaacgacctacaccgaactgagatacctacagcgtgagctatgagaaagcgccacgcttcccgaagggagaaaggcggacaggtatcccgtaagcggcagggtcggaacaggagagcgcacgagggagcttccagggggaaacgcctggtatctttatagtcctgtcgggtttcgccacctctgacttgagcgtcgatttttgtgatgctcgtcaggggggcggagcctatggaaaaacgccagcaacgcggcctttttacggttcctggccttttgctggccttttgctcttcgattaaccctagaaagatagtctgcgtaaaattgacgcatgtctagacatcttggaccattagctccacaggtatcttcttccctctagtggtcataacagcagcttcagctacctctctctctgctgccagtagagggcacacttactttactcattcctttaatggtcttttctggacaccactaggggtcagaagtagttcatcaaactttcttccctccctagctagcgacattgattattgactagttattattagtaatcaattacggggtcattagttcatagcccatatatggagttccgcgttacataacttacggtaaatggcccgcctggctgaccgcccaacgacccccgcccattgacgtcaataatgacgtatgttcccatagtaacgccaatagggactttccattgacgtcaatgggtggagtatttacggtaaactgcccacttggcagtacatcaagtgtatcatatgccaagtacgccccctattgacgtcaatgacggtaaatggcccgcctggcattatgcccagtacatgaccttatgggactttcctacttggcagtacatctacgtattagtcatcgctattaccatgcgatcgaaaagtgccttcaaagaatcccaccagaatggcacaggtgggcataatgggtctgtctcatcgtcaaaggacccaaggagtctaaaggaaactctaactacaacacccaaatgccacaaaaccttagttatatatacaaactatcatccctgcctatctgtcaccatctcatctataaaaacttgtgaaaatacgtaatcctcaggagacttcaattaggtataaataccagcagccagaggaggtgcagaagcttcgaggggctcgcatctctccttcacgcgcccgccgccctacctgaggccgccatccacgccggttgagtcgcgttctgccgcctcccgcctgtggtgcctcctgaactgcgtccgccgtctaggtaagtttaaagctcaggtcgagaccgggcctttgtccggcgctcccttggagcctacctagactcagccggctctccacgctttgcctgaccctgcttgctcaactctacgtctttgtttcgttttctgttctgcgccgttacagatccaagctgtgaccggcgcctacgaattcgccaccatggaggccccagctcagctgctgttcctgctgctgctgtggctgccagacaccacaggagaggtgcagctggtggagagcggcggcggcctggtgcagcccggcggcagcctgagactgagctgcgccgccagcggcagacccttcagcatctacgacatgggctggttcagacaggcccccgacaaggagagagagagcgtggccgtgatcaacctggccagaggcaacacctactacgccgacagcgtgaagggcagattcaccatcagcagagacaacgccaagaacaccgtgtacctccagatgaacagcctgagagccgaggacaccgccgtgtacagctgcggcgtggacagaagacagtacggcctgggcatcccccccctggccgaccactggggccagggcacccaggtgaccgtgagcagctgataag

SEQ ID NO: 46 - DNA, 3045 bp, synthetic construct
  source 1..3045: mol_type = other DNA
cttaaggtgcgccttatagtgcggaaaatacggtataagatctaatcagcagttcaacctgttgatagtatgtactaagctctcatgtttaatgtactaagctctcatgtttaatgaactaaaccctcatggctaatgtactaagctctcatggctaatgtactaagctctcatgtttcatgtactaagctctcatgtttgaacaataaaattaatataaatcagcaacttaaatagcctctaaggttttaagttttataagaaaaaaaagaatatataaggcttttaaaggttttaaggtttcctagctttaggttctgcttttctcaataacctctttggctgaagtgtattcctcaagaggttcttctgccattgcttgttcaataactctcagtattggttctgggatatctgaaggggttgataacaaatattcaattgcttccagagtaggctcatcaatatcagaactcacttttctgatgatctccaattttctttcatctgttgacatgatggccctcctatagtgagttgtattatactatgcagatatactatgccaatgtttaattgtcaacctgcaggaatataccgtattttccgcactataaggcgcacctctagacatcttggaccattagctccacaggtatcttcttccctctagtggtcataacagcagcttcagctacctctctctctgctgccagtagagggcacacttactttactcattcctttaatggtcttttctggacaccactaggggtcagaagtagttcatcaaactttcttccctccctagctagcggtgtggaaagtccccaggctccccagcaggcagaagtatgcaaagcatgcatctcaattagtcagcaaccaggtgtggaaagtccccaggctccccagcaggcagaagtatgcaaagcatgcatctcaattagtcagcaaccaaggatctgcgatcgctccggtgcccgtcagtgggcagagcgcacatcgcccacagtccccgagaagttggggggaggggtcggcaattgaacgggtgcctagagaaggtggcgcggggtaaactgggaaagtgatgtcgtgtactggctccgcctttttcccgagggtgggggagaaccgtatataagtgcagtagtcgccgtgaacgttctttttcgcaacgggtttgccgccagaacacagctgaagcttcgaggggctcgcatctctccttcacgcgcccgccgccctacctgaggccgccatccacgccggttgagtcgcgttctgccgcctcccgcctgtggtgcctcctgaactgcgtccgccgtctaggtaagtttatagctcaggtcgagaccgggcctttgtccggcgctcccttggagcctacctagactcagccggctctccacgctttgcctgaccctgcttgctcaactctacgtctttgtttcgttttctgttctgcgccgttacagatccaagctgtgaccggcgcctacgaattcgccaccatggccttaccagtgaccgccttgctcctgccgctggccttgctgctccacgccgccaggccgagccaggtgcaggtggtggagagcggcggcggcttcgtgcaggccggcggcagcctgcgcctgagctgcgccgccagcacccccatcatcagcatcgcctacatgggctggtaccgccagatcagcgagaaggagcgccagctggtggccaccatcaacagcggcggcaagacctactacgccgacagcgtgaagggccgcttcaccatcagccgcgacaacgccaagaacaccctgtacctgcagatgaacatgctgaagcccgaggacaccggcatgtactactgcgccgccagcaacaaggactacaacgactacgaccccgactggggccagggcacccaggtgaccgtgagcagcttcgtgccggtcttcctgccagcgaagcccaccacgacgccagcgccgcgaccaccaacaccggcgcccaccatcgcgtcgcagcccctgtccctgcgcccagaggcgtgccggccagcggcggggggcgcagtgcacacgagggggctggacttcgcctgtgatcccttttgggtgctggtggtggttggtggagtcctggcttgctatagcttgctagtaacagtggcctttattattttctgggtgaggagtaagaggagcaggctcctgcacagtgactacatgaacatgactccccgccgccccgggcccacccgcaagcattaccagccctatgccccaccacgcgacttcgcagcctatcgctccagagtgaagttcagcaggagcgcagacgcccccgcgtaccagcagggccagaaccagctctataacgagctcaatctaggacgaagagaggagtacgatgttttggacaagagacgtggccgggaccctgagatggggggaaagccgagaaggaagaaccctcaggaaggcctgtacaatgaactgcagaaagataagatggcggaggcctacagtgagattgggatgaaaggcgagcgccggaggggcaaggggcacgatggcctttaccagggtctcagtacagccaccaaggacacctacgacgcccttcacatgcaggccctgccccctcgctgataagtcgacctgtgccttctagttgccagccatctgttgtttgcccctcccccgtgccttccttgaccctggaaggtgccactcccactgtcctttcctaataaaatgaggaaattgcatcgcattgtctgagtaggtgtcattctattctggggggtggggtggggcaggacagcaagggggaggattgggatgacaatagcaggcatgctggggatgcggtgggctctatgggatatcaataaaatatctttattttcattacatctgtgtgttggttttttgtgtgaatcagtatgactaacatacgctctccatcaaaacaaaacgaaacaaaacaaactagcaaaataggctgtccccagtgcaagtgcaggtgccagaacatttctct

SEQ ID NO: 47 - DNA, 2622 bp, synthetic construct
  source 1..2622: mol_type = other DNA
aatcagcagttcaacctgttgatagtatgtactaagctctcatgtttaatgtactaagctctcatgtttaatgaactaaaccctcatggctaatgtactaagctctcatggctaatgtactaagctctcatgtttcatgtactaagctctcatgtttgaacaataaaattaatataaatcagcaacttaaatagcctctaaggttttaagttttataagaaaaaaaagaatatataaggcttttaaaggttttaaggtttcctagctttaggttctgcttttctcaataacctctttggctgaagtgtattcctcaagaggttcttctgccattgcttgttcaataactctcagtattggttctgggatatctgaaggggttgataacaaatattcaattgcttccagagtaggctcatcaatatcagaactcacttttctgatgatctccaattttctttcatctgttgacatgatggccctcctatagtgagttgtattatactatgcagatatactatgccaatgtttaattgtcaacctgcaggaatataccgtattttccgcactataaggcgcacctctagacatcttggaccattagctccacaggtatcttcttccctctagtggtcataacagcagcttcagctacctctctctctgctgccagtagagggcacacttactttactcattcctttaatggtcttttctggacaccactaggggtcagaagtagttcatcaaactttcttccctccctagctagcgacattgattattgactagttattattagtaatcaattacggggtcattagttcatagcccatatatggagttccgcgttacataacttacggtaaatggcccgcctggctgaccgcccaacgacccccgcccattgacgtcaataatgacgtatgttcccatagtaacgccaatagggactttccattgacgtcaatgggtggagtatttacggtaaactgcccacttggcagtacatcaagtgtatcatatgccaagtacgccccctattgacgtcaatgacggtaaatggcccgcctggcattatgcccagtacatgaccttatgggactttcctacttggcagtacatctacgtattagtcatcgctattaccatgcgatcgaaaagtgccttcaaagaatcccaccagaatggcacaggtgggcataatgggtctgtctcatcgtcaaaggacccaaggagtctaaaggaaactctaactacaacacccaaatgccacaaaaccttagttatatatacaaactatcatccctgcctatctgtcaccatctcatctataaaaacttgtgaaaatacgtaatcctcaggagacttcaattaggtataaataccagcagccagaggaggtgcagaagcttcgaggggctcgcatctctccttcacgcgcccgccgccctacctgaggccgccatccacgccggttgagtcgcgttctgccgcctcccgcctgtggtgcctcctgaactgcgtccgccgtctaggtaagtttaaagctcaggtcgagaccgggcctttgtccggcgctcccttggagcctacctagactcagccggctctccacgctttgcctgaccctgcttgctcaactctacgtctttgtttcgttttctgttctgcgccgttacagatccaagctgtgaccggcgcctacgtcgagaagacaggaattgccaccatggaggccccagctcagctgctgttcctgctgctgctgtggctgccagacaccacaggagaggtgcagctggtggagagcggcggcggcctggtgcagcccggcggcagcctgagactgagctgcgccgccagcggcagacccttcagcatctacgacatgggctggttcagacaggcccccgacaaggagagagagagcgtggccgtgatcaacctggccagaggcaacacctactacgccgacagcgtgaagggcagattcaccatcagcagagacaacgccaagaacaccgtgtacctccagatgaacagcctgagagccgaggacaccgccgtgtacagctgcggcgtggacagaagacagtacggcctgggcatcccccccctggccgaccactggggccagggcacccaggtgaccgtgagcagctgataaggatcctgcactagtgctgtcgacctgtgccttctagttgccagccatctgttgtttgcccctcccccgtgccttccttgaccctggaaggtgccactcccactgtcctttcctaataaaatgaggaaattgcatcgcattgtctgagtaggtgtcattctattctggggggtggggtggggcaggacagcaagggggaggattgggatgacaatagcaggcatgctggggatgcggtgggctctatgggatatcaataaaatatctttattttcattacatctgtgtgttggttttttgtgtgaatcagtatgactaacatacgctctccatcaaaacaaaacgaaacaaaacaaactagcaaaataggctgtccccagtgcaagtgcaggtgccagaacatttctctcttaaggtgcgccttatagtgcggaaaatacggtataagatct

SEQ ID NO: 48 - DNA, 4467 bp, synthetic construct
  source 1..4467: mol_type = other DNA
cctgtgccttctagttgccagccatctgttgtttgcccctcccccgtgccttccttgaccctggaaggtgccactcccactgtcctttcctaataaaatgaggaaattgcatcgcattgtctgagtaggtgtcattctattctggggggtggggtggggcaggacagcaagggggaggattgggatgacaatagcaggcatgctggggatgcggtgggctctatgggatatcaataaaatatctttattttcattacatctgtgtgttggttttttgtgtgaatcagtatgactaacatacgctctccatcaaaacaaaacgaaacaaaacaaactagcaaaataggctgtccccagtgcaagtgcaggtgccagaacatttctctcttaagcatgcgtcaattttacgcatgattatctttaacgtacgtcacaatatgattatctttctagggttaaggcgcgcccatgcatgggaggagaccgggacgagacgaaccctgataaatgcttcaataatattatgattgaacaagatggattgcacgcaggttctccggccgcttgggtggagaggctattcggctatgactgggcacaacagacaatcggctgctctgatgccgccgtgttccggctgtcagcgcaggggcgcccggttctttttgtcaagaccgacctgtccggtgccctgaatgaactgcaagacgaggcagcgcggctatcgtggctggccacgacgggcgttccttgcgcagctgtactcgacgttgtcactgaagcgggaagggactggctgctattgggcgaagtgccggggcaggatctcctgtcatctcaccttgctcctgccgagaaagtatccatcatggctgatgcaatgcggcggctgcatacgcttgatccggctacctgcccattcgaccaccaagcgaaacatcgcatcgagagagcacgtactcggatggaagccggtcttgtcgatcaggatgatctggacgaagagcatcaggggctcgcgccagccgaactgttcgccaggctcaaggcgagcatgcccgacggcgaggatctcgtcgtgacccatggcgatgcctgcttgccgaatatcatggtggaaaatggccgcttttctggattcatcgactgtggccggctgggtgtggcggaccgctatcaggacatagcgttggctacccgtgatattgctgaagagcttggcggcgaatgggctgaccgcttcctcgtgctttacggtatcgccgctcccgattcgcagcgcatcgccttctatcgccttcttgacgagttcttctgagacggcatgaccaaaatccccgtgagttttcgttccactgagcgtcagaccccgtagaaaagatcaaaggatcttcttgagatcctttttttctgcgcgtaatctgctgcttgcaaacaaaaaaaccaccgctaccagcggtggtttgtttgccggatcaagagctaccaactctttttccgaaggtaactggcttcagcagagcgcagataccaaatactgttcttctagtgtagccgtagttaggccaccacttcaagaactctgtagcaccgcctacatacctcgctctgctaatcctgttaccagtggctgctgccagtggcgataagtcgtgtcttaccgggttggactcaagacgatagttaccggataaggcgcagcggtcgggctgaacggggggttcgtgcacacagcccagcttggagcgaacgacctacaccgaactgagatacctacagcgtgagctatgagaaagcgccacgcttcccgaagggagaaaggcggacaggtatcccgtaagcggcagggtcggaacaggagagcgcacgagggagcttccagggggaaacgcctggtatctttatagtcctgtcgggtttcgccacctctgacttgagcgtcgatttttgtgatgctcgtcaggggggcggagcctatggaaaaacgccagcaacgcggcctttttacggttcctggccttttgctggccttttgctcttcgattaaccctagaaagatagtctgcgtaaaattgacgcatgtctagacatcttggaccattagctccacaggtatcttcttccctctagtggtcataacagcagcttcagctacctctctctctgctgccagtagagggcacacttactttactcattcctttaatggtcttttctggacaccactaggggtcagaagtagttcatcaaactttcttccctccctagctagcggtgtggaaagtccccaggctccccagcaggcagaagtatgcaaagcatgcatctcaattagtcagcaaccaggtgtggaaagtccccaggctccccagcaggcagaagtatgcaaagcatgcatctcaattagtcagcaaccaaggatctgcgatcgctccggtgcccgtcagtgggcagagcgcacatcgcccacagtccccgagaagttggggggaggggtcggcaattgaacgggtgcctagagaaggtggcgcggggtaaactgggaaagtgatgtcgtgtactggctccgcctttttcccgagggtgggggagaaccgtatataagtgcagtagtcgccgtgaacgttctttttcgcaacgggtttgccgccagaacacagctgaagcttcgaggggctcgcatctctccttcacgcgcccgccgccctacctgaggccgccatccacgccggttgagtcgcgttctgccgcctcccgcctgtggtgcctcctgaactgcgtccgccgtctaggtaagtttatagctcaggtcgagaccgggcctttgtccggcgctcccttggagcctacctagactcagccggctctccacgctttgcctgaccctgcttgctcaactctacgtctttgtttcgttttctgttctgcgccgttacagatccaagctgtgaccggcgcctacgaattcgccaccatggccttaccagtgaccgccttgctcctgccgctggccttgctgctccacgccgccaggccgagcaagggcgaggagctgttcaccggggtggtgcccatcctggtcgagctggacggcgacgtaaacggccacaagttcagcgtgtccggcgagggcgagggcgatgccacctacggcaagctgaccctgaagttcatctgcaccaccggcaagctgcccgtgccctggcccaccctcgtgaccaccctgacctacggcgtgcagtgcttcagccgctaccccgaccacatgaagcagcacgacttcttcaagtccgccatgcccgaaggctacgtccaggagcgcaccatcttcttcaaggacgacggcaactacaagacccgcgccgaggtgaagttcgagggcgacaccctggtgaaccgcatcgagctgaagggcatcgacttcaaggaggacggcaacatcctggggcacaagctggagtacaactacaacagccacaacgtctatatcatggccgacaagcagaagaacggcatcaaggtgaacttcaagatccgccacaacatcgaggacggcagcgtgcagctcgccgaccactaccagcagaacacccccatcggcgacggccccgtgctgctgcccgacaaccactacctgagcacccagtccgccctgagcaaagaccccaacgagaagcgcgatcacatggtcctgctggagttcgtgaccgccgccgggatcactctcggcatggacgagctgtacaagttcgtgccggtcttcctgccagcgaagcccaccacgacgccagcgccgcgaccaccaacaccggcgcccaccatcgcgtcgcagcccctgtccctgcgcccagaggcgtgccggccagcggcggggggcgcagtgcacacgagggggctggacttcgcctgtgatcccttttgggtgctggtggtggttggtggagtcctggcttgctatagcttgctagtaacagtggcctttattattttctgggtgaggagtaagaggagcaggctcctgcacagtgactacatgaacatgactccccgccgccccgggcccacccgcaagcattaccagccctatgccccaccacgcgacttcgcagcctatcgctccagagtgaagttcagcaggagcgcagacgcccccgcgtaccagcagggccagaaccagctctataacgagctcaatctaggacgaagagaggagtacgatgttttggacaagagacgtggccgggaccctgagatggggggaaagccgagaaggaagaaccctcaggaaggcctgtacaatgaactgcagaaagataagatggcggaggcctacagtgagattgggatgaaaggcgagcgccggaggggcaaggggcacgatggcctttaccagggtctcagtacagccaccaaggacacctacgacgcccttcacatgcaggccctgccccctcgctgataagtcga

SEQ ID NO: 49 - protein, 50 aa, synthetic construct
MSTDERKLEIIRKVSSDIDEPTLEAIEYLLSTPSDIPEPILRVIEQAMAE

SEQ ID NO: 50 - protein, 69 aa, synthetic construct
MPKKATNLSLNSELLAEAKRLNINLSATMEKALEKEVRQRLKTEWLKQNAEGINACNELTENHGLFSDS

SEQ ID NO: 51 - protein, 60 aa, synthetic construct
MSTDERKLEIIRKVSSDIDEPTLEAIEYLLSTPSDIPEPILRVIEQAMAEEPLEEYTSAK

SEQ ID NO: 52 - protein, 68 aa, synthetic construct
MSTDERKLEIIRKVSSDIDEPTLEAIEYLLSTPSDIPEPILRVIEQAMAEEPLEEYTSAKEVIEKSRT

SEQ ID NO: 53 - protein, 73 aa, synthetic construct
MPKKATNLSLNSELLAEAKRLNINLSATMEKALEKEVRQRLKTEWLKQNAEGINACNELTENHGLFSDSYRVF

SEQ ID NO: 54 - protein, 77 aa, synthetic construct
MRNAYSTQAPKKATNLSLNSELLAEAKRLNINLSATMEKALEKEVRQRLKTEWLKQNAEGINACNELTENHGLFSDS

SEQ ID NO: 55 - protein, 81 aa, synthetic construct
MRNAYSTQAPKKATNLSLNSELLAEAKRLNINLSATMEKALEKEVRQRLKTEWLKQNAEGINACNELTENHGLFSDSYRVF

SEQ ID NO: 56 - DNA, 207 bp, synthetic construct
  source 1..207: mol_type = other DNA
atgtcaacagatgaaagaaaattggagatcatcagaaaagtgagttctgatattgatgagcctactctggaagcaattgaatatttgttatcaaccccttcagatatcccagaaccaatactgagagttattgaacaagcaatggcagaagaacctcttgaggaatacacttcagccaaagaggttattgagaaaagcagaacctaa

SEQ ID NO: 57 - DNA, 246 bp, synthetic construct
  source 1..246: mol_type = other DNA
atgagaaatgcatatagtacccaagcaccaaagaaagctacaaacctgagcttaaacagtgagttacttgcagaggctaaaagattaaatataaaccttagtgcaacaatggaaaaggcacttgaaaaagaagtaagacaaagactgaagactgaatggttaaagcaaaatgctgagggcattaatgcttgtaatgagctaactgaaaatcatggactattttctgattcttacagagtattctaa

SEQ ID NO: 58 - DNA, 267 bp, synthetic construct
  source 1..267: mol_type = other DNA
aatcagcagttcaacctgttgatagtatgtactaagctctcatgtttaatgtactaagctctcatgtttaatgaactaaaccctcatggctaatgtactaagctctcatggctaatgtactaagctctcatgtttcatgtactaagctctcatgtttgaacaataaaattaatataaatcagcaacttaaatagcctctaaggttttaagttttataagaaaaaaaagaatatataaggcttttaaaggttttaaggtttcctagct

SEQ ID NO: 59 - DNA, 559 bp, synthetic construct
  source 1..559: mol_type = other DNA
gaattcttaattaaaatcagcagttcaacctgttgatagtatgtactaagctctcatgtttaatgtactaagctctcatgtttaatgaactaaaccctcatggctaatgtactaagctctcatggctaatgtactaagctctcatgtttcatgtactaagctctcatgtttgaacaataaaattaatataaatcagcaacttaaatagcctctaaggttttaagttttataagaaaaaaaagaatatataaggcttttaaaggttttaaggtttcctagctttaggttctgcttttctcaataacctctttggctgaagtgtattcctcaagaggttcttctgccattgcttgttcaataactctcagtattggttctgggatatctgaaggggttgataacaaatattcaattgcttccagagtaggctcatcaatatcagaactcacttttctgatgatctccaattttctttcatctgttgacatgatggccctcctatagtgagttgtattatactatgcagatatactatgccaatgtttaattgtcaactagt

SEQ ID NO: 60 - DNA, 592 bp, synthetic construct
  source 1..592: mol_type = other DNA
ttaattaaaatcagcagttcaacctgttgatagtatgtactaagctctcatgtttaatgtactaagctctcatgtttaatgaactaaaccctcatggctaatgtactaagctctcatggctaatgtactaagctctcatgtttcatgtactaagctctcatgtttgaacaataaaattaatataaatcagcaacttaaatagcctctaaggttttaagttttataagaaaaaaaagaatatataaggcttttaaaggttttaaggtttcctagctttagaatactctgtaagaatcagaaaatagtccatgattttcagttagctcattacaagcattaatgccctcagcattttgctttaaccattcagtcttcagtctttgtcttacttctttttcaagtgccttttccattgttgcactaaggtttatatttaatcttttagcctctgcaagtaactcactgtttaagctcaggtttgtagctttctttggtgcttgggtactatatgcatttctcatgatggccctcctatagtgagttgtattatactatgcagatatactatgccaatgtttaattgtcaactagt

SEQ ID NO: 61 - DNA, 3720 bp, synthetic construct
  source 1..3720: mol_type = other DNA
tcgaagagcaaaaggccagcaaaaggccaggaaccgtaaaaaggccgcgttgctggcgtttttccataggctccgcccccctgacgagcatcacaaaaatcgacgctcaagtcagaggtggcgaaacccgacaggactataaagataccaggcgtttccccctggaagctccctcgtgcgctctcctgttccgaccctgccgcttacgggatacctgtccgcctttctcccttcgggaagcgtggcgctttctcatagctcacgctgtaggtatctcagttcggtgtaggtcgttcgctccaagctgggctgtgtgcacgaaccccccgttcagcccgaccgctgcgccttatccggtaactatcgtcttgagtccaacccggtaagacacgacttatcgccactggcagcagccactggtaacaggattagcagagcgaggtatgtaggcggtgctacagagttcttgaagtggtggcctaactacggctacactagaagaacagtatttggtatctgcgctctgctgaagccagttaccttcggaaaaagagttggtagctcttgatccggcaaacaaaccaccgctggtagcggtggtttttttgtttgcaagcagcagattacgcgcagaaaaaaaggatctcaagaagatcctttgatcttttctacggggtctgacgctcagtggaacgaaaactcacggggattttggtcatgccgtctcagaagaactcgtcaagaaggcgatagaaggcgatgcgctgcgaatcgggagcggcgataccgtaaagcacgaggaagcggtcagcccattcgccgccaagctcttcagcaatatcacgggtagccaacgctatgtcctgatagcggtccgccacacccagccggccacagtcgatgaatccagaaaagcggccattttccaccatgatattcggcaagcaggcatcgccatgggtcacgacgagatcctcgccgtcgggcatgctcgccttgagcctggcgaacagttcggctggcgcgagcccctgatgctcttcgtccagatcatcctgatcgacaagaccggcttccatccgagtacgtgctctctcgatgcgatgtttcgcttggtggtcgaatgggcaggtagccggatcaagcgtatgcagccgccgcattgcatcagccatgatggatactttctcggcaggagcaaggtgagatgacaggagatcctgccccggcacttcgcccaatagcagccagtcccttcccgcttcagtgacaacgtcgagtacagctgcgcaaggaacgcccgtcgtggccagccacgatagccgcgctgcctcgtcttgcagttcattcagggcaccggacaggtcggtcttgacaaaaagaaccgggcgcccctgcgctgacagccggaacacggcggcatcagagcagccgattgtctgttgtgcccagtcatagccgaatagcctctccacccaagcggccggagaacctgcgtgcaatccatcttgttcaatcataatattattgaagcatttatcagggttcgtctcgtcccggtctcctccctataccgtattttccgcactataaggcgcaccccgtattttccgcactataaggcgcacctctagacatcttggaccattagctccacaggtatcttcttccctctagtggtcataacagcagcttcagctacctctctctctgctgccagtagagggcacacttactttactcattcctttaatggtcttttctggacaccactaggggtcagaagtagttcatcaaactttcttccctccctagctagcggtgtggaaagtccccaggctccccagcaggcagaagtatgcaaagcatgcatctcaattagtcagcaaccaggtgtggaaagtccccaggctccccagcaggcagaagtatgcaaagcatgcatctcaattagtcagcaaccaaggatctgcgatcgctccggtgcccgtcagtgggcagagcgcacatcgcccacagtccccgagaagttggggggaggggtcggcaattgaacgggtgcctagagaaggtggcgcggggtaaactgggaaagtgatgtcgtgtactggctccgcctttttcccgagggtgggggagaaccgtatataagtgcagtagtcgccgtgaacgttctttttcgcaacgggtttgccgccagaacacagctgaagcttcgaggggctcgcatctctccttcacgcgcccgccgccctacctgaggccgccatccacgccggttgagtcgcgttctgccgcctcccgcctgtggtgcctcctgaactgcgtccgccgtctaggtaagtttatagctcaggtcgagaccgggcctttgtccggcgctcccttggagcctacctagactcagccggctctccacgctttgcctgaccctgcttgctcaactctacgtctttgtttcgttttctgttctgcgccgttacagatccaagctgtgaccggcgcctacgaattgccaccatggtgagcaagggagaggagctgttcactggggtggtgcccatcctggtggagctggatggagatgtgaatggccacaagttctctgtgtctggagagggagagggagatgccacctatggcaagctgaccctgaagttcatctgcaccacaggcaagctgcctgtgccctggcccaccctggtgaccaccctgacctatggagtgcagtgcttcagcagataccctgaccacatgaagcagcatgacttcttcaagtctgccatgcctgagggctatgtccaggagagaaccatcttcttcaaggatgatggcaactacaagaccagagctgaggtgaagtttgagggagacaccctggtgaacagaattgagctgaagggcattgacttcaaggaggatggcaacatcctggggcacaagctggagtacaactacaacagccacaatgtctatatcatggctgacaagcagaagaatggcatcaaggtgaacttcaagatcagacacaacattgaggatggctctgtgcagctggctgaccactaccagcagaacacccccattggagatggccctgtgctgctgcctgacaaccactacctgagcacccagtctgccctgagcaaggaccccaatgagaagagagatcacatggtcctgctggagtttgtgacagctgctgggatcactctgggcatggatgagctgtacaagtaaggatcctgcactagtgctgtcgacctgtgccttctagttgccagccatctgttgtttgcccctcccccgtgccttccttgaccctggaaggtgccactcccactgtcctttcctaataaaatgaggaaattgcatcgcattgtctgagtaggtgtcattctattctggggggtggggtggggcaggacagcaagggggaggattgggatgacaatagcaggcatgctggggatgcggtgggctctatgggatatcaataaaatatctttattttcattacatctgtgtgttggttttttgtgtgaatcagtatgactaacatacgctctccatcaaaacaaaacgaaacaaaacaaactagcaaaataggctgtccccagtgcaagtgcaggtgccagaacatttctctcttaaggtgcgccttatagtgcggaaaatacggggtgcgccttatagtgcggaaaatacggtataagatct